European Patent Application EP 4 124 348 A1, published February 1, 2023. Title: NANOPARTICLES FOR CELL DELIVERY. Applicant: 4basebio Discovery Limited. The sequence listing filed with the application follows.

SEQUENCE LISTING (43 sequences)

SEQ ID NO: 1 - protein, 7 aa, Artificial Sequence
  Artificial Sequence
YGLPHKF

SEQ ID NO: 2 - protein, 9 aa, Artificial Sequence
  Artificial Sequence
CYGLPHKFC

SEQ ID NO: 3 - protein, 11 aa, Artificial Sequence
  Artificial Sequence
GACYGLPHKFC

SEQ ID NO: 4 - protein, 27 aa, Artificial Sequence
  Artifical Sequence
KKKKKKKKKKKKKKKKGACYGLPHKFC

SEQ ID NO: 5 - protein, 41 aa, Artificial Sequence
  Artificial Sequence
KKKKKKKKKKKKKKKKKKKKKKKKKKKKKKGACYGLPHKFC

SEQ ID NO: 6 - protein, 7 aa, Artificial Sequence
  Artifical Sequence
ASSLNIA

SEQ ID NO: 7 - protein, 12 aa, Artificial Sequence
  Artifical Sequence
RRQPPRSISSHP

SEQ ID NO: 8 - protein, 12 aa, Artificial Sequence
  Artifical Sequence
SKTFNTHPQSTP

SEQ ID NO: 9 - protein, 9 aa, Artificial Sequence
  Artifical Sequence
CASSLNIAC

SEQ ID NO: 10 - protein, 11 aa, Artificial Sequence
  Artifical Sequence
GACASSLNIAC

SEQ ID NO: 11 - protein, 15 aa, Artificial Sequence
  Artifical Sequence
RVRRGACASSLNIAC

SEQ ID NO: 12 - protein, 31 aa, Artificial Sequence
  Artifical Sequence
KKKKKKKKKKKKKKKKRVRRGACASSLNIAC

SEQ ID NO: 13 - protein, 45 aa, Artificial Sequence
  Artifical Sequence
KKKKKKKKKKKKKKKKKKKKKKKKKKKKKKRVRRGACASSLNIAC

SEQ ID NO: 14 - protein, 27 aa, Artificial Sequence
  Artifical Sequence
KKKKKKKKKKKKKKKKGACASSLNIAC

SEQ ID NO: 15 - protein, 41 aa, Artificial Sequence
  Artifical Sequence
KKKKKKKKKKKKKKKKKKKKKKKKKKKKKKGACASSLNIAC

SEQ ID NO: 16 - protein, 9 aa, Artificial Sequence
  Artifical Sequence
GAASSLNIA

SEQ ID NO: 17 - protein, 25 aa, Artificial Sequence
  Artifical Sequence
KKKKKKKKKKKKKKKKGAASSLNIA

SEQ ID NO: 18 - protein, 39 aa, Artificial Sequence
  Artifical Sequence
KKKKKKKKKKKKKKKKKKKKKKKKKKKKKKGAASSLNIA

SEQ ID NO: 19 - protein, 14 aa, Artificial Sequence
  Artifical Sequence
CRRQPPRSISSHPC

SEQ ID NO: 20 - protein, 16 aa, Artificial Sequence
  Artifical Sequence
GACRRQPPRSISSHPC

SEQ ID NO: 21 - protein, 20 aa, Artificial Sequence
  Artifical Sequence
RVRRGACRRQPPRSISSHPC

SEQ ID NO: 22 - protein, 36 aa, Artificial Sequence
  Artifical Sequence
KKKKKKKKKKKKKKKKRVRRGACRRQPPRSISSHPC

SEQ ID NO: 23 - protein, 50 aa, Artificial Sequence
  Artifical Sequence
KKKKKKKKKKKKKKKKKKKKKKKKKKKKKKRVRRGACRRQPPRSISSHPC

SEQ ID NO: 24 - protein, 32 aa, Artificial Sequence
  Artifical Sequence
KKKKKKKKKKKKKKKKGACRRQPPRSISSHPC

SEQ ID NO: 25 - protein, 46 aa, Artificial Sequence
  Artifical Sequence
KKKKKKKKKKKKKKKKKKKKKKKKKKKKKKGACRRQPPRSISSHPC

SEQ ID NO: 26 - protein, 14 aa, Artificial Sequence
  Artifical Sequence
GARRQPPRSISSHP

SEQ ID NO: 27 - protein, 30 aa, Artificial Sequence
  Artifical Sequence
KKKKKKKKKKKKKKKKGARRQPPRSISSHP

SEQ ID NO: 28 - protein, 44 aa, Artificial Sequence
  Artifical Sequence
KKKKKKKKKKKKKKKKKKKKKKKKKKKKKKGARRQPPRSISSHP

SEQ ID NO: 29 - protein, 14 aa, Artificial Sequence
  Artifical Sequence
CSKTFNTHPQSTPC

SEQ ID NO: 30 - protein, 16 aa, Artificial Sequence
  Artifical Sequence
GACSKTFNTHPQSTPC

SEQ ID NO: 31 - protein, 20 aa, Artificial Sequence
  Artifical Sequence
RVRRGACSKTFNTHPQSTPC

SEQ ID NO: 32 - protein, 36 aa, Artificial Sequence
  Artifical Sequence
KKKKKKKKKKKKKKKKRVRRGACSKTFNTHPQSTPC

SEQ ID NO: 33 - protein, 50 aa, Artificial Sequence
  Artifical Sequence
KKKKKKKKKKKKKKKKKKKKKKKKKKKKKKRVRRGACSKTFNTHPQSTPC

SEQ ID NO: 34 - protein, 32 aa, Artificial Sequence
  Artifical Sequence
KKKKKKKKKKKKKKKKGACSKTFNTHPQSTPC

SEQ ID NO: 35 - protein, 46 aa, Artificial Sequence
  Artifical Sequence
KKKKKKKKKKKKKKKKKKKKKKKKKKKKKKGACSKTFNTHPQSTPC

SEQ ID NO: 36 - protein, 14 aa, Artificial Sequence
  Artifical Sequence
GASKTFNTHPQSTP

SEQ ID NO: 37 - protein, 30 aa, Artificial Sequence
  Artifical Sequence
KKKKKKKKKKKKKKKKGASKTFNTHPQSTP

SEQ ID NO: 38 - protein, 44 aa, Artificial Sequence
  Artifical Sequence
KKKKKKKKKKKKKKKKKKKKKKKKKKKKKKGASKTFNTHPQSTP

SEQ ID NO: 39 - protein, 4 aa, Artificial Sequence
  Artifical Sequence
RVRR

SEQ ID NO: 40 - protein, 5 aa, Artificial Sequence
  Artificial Sequence
  misc_feature (1)..(3): Xaa is c-aminocaproic acid
  misc_feature (3)..(3): Xaa is c-aminocaproic acid
XSXGG

SEQ ID NO: 41 - protein, 5 aa, Artificial Sequence
  Artificial Sequence
  misc_feature (1)..(1): Xaa is c-aminocaproic acid
  misc_feature (3)..(3): Xaa is c-aminocaproic acid
XSXGA

SEQ ID NO: 42 - DNA, 13 bp, Artificial Sequence
  Artificial Sequence
aaaaaacataaaa

SEQ ID NO: 43 - protein, 5 aa, Artificial Sequence
  Artificial Sequence
  misc_feature (1)..(1): Xaa is c-aminocaproic acid
  misc_feature (3)..(3): Xaa is c-aminocaproic acid
XSXAA